European Patent Specification EP 3 876 922 B1, published February 25, 2026. Title: EXPLOITING ESTROGEN RECEPTOR BETA AND TP53 INTERACTION AS A NEW THERAPEUTIC STRATEGY FOR CANCER. Applicant: Health Research, Inc. Das, Gokul M. The sequence listing filed with the application follows.

SEQUENCE LISTING (42 sequences)

SEQ ID NO: 1 - DNA, 43 bp, Artificial Sequence
  Synthetic sequence
ccatagcggccgccaccatggatataaaaactcaccatctagc

SEQ ID NO: 2 - DNA, 91 bp, Artificial Sequence
  Synthetic sequence
ggtcaacgcgttcaagcgtaatctggaacatcgtatgggtaagcgtaatctggaacatcgtatgggtactgagactgtgggttctgggagc

SEQ ID NO: 3 - DNA, 24 bp, Artificial Sequence
  Synthetic sequence
cctatgtagacagccaccatgaat

SEQ ID NO: 4 - DNA, 24 bp, Artificial Sequence
  Synthetic sequence
cccacctcccaagttagtgacatt

SEQ ID NO: 5 - DNA, 22 bp, Artificial Sequence
  Synthetic sequence
gctttggtttgggtgattgcca

SEQ ID NO: 6 - DNA, 21 bp, Artificial Sequence
  Synthetic sequence
cgttcaagcgtaatctggaac

SEQ ID NO: 7 - DNA, 21 bp, Artificial Sequence
  Synthetic sequence
cgatgctttggtttgggtgat

SEQ ID NO: 8 - DNA, 21 bp, Artificial Sequence
  Synthetic sequence
gccctctttgcttttactgtc

SEQ ID NO: 9 - DNA, 21 bp, Artificial Sequence
  Synthetic sequence
ctttaggccaccgagttgatt

SEQ ID NO: 10 - DNA, 23 bp, Artificial Sequence
  Synthetic sequence
atgggtcagaaggattcctatgt

SEQ ID NO: 11 - DNA, 22 bp, Artificial Sequence
  Synthetic sequence
aaggtctcaaacatgatctggg

SEQ ID NO: 12 - DNA, 22 bp, Artificial Sequence
  Synthetic sequence
gagactctcagggtcgaaaacg

SEQ ID NO: 13 - DNA, 20 bp, Artificial Sequence
  Synthetic sequence
gatgtagagcgggcctttga

SEQ ID NO: 14 - DNA, 20 bp, Artificial Sequence
  Synthetic sequence
atgcctgcctcaccttcatc

SEQ ID NO: 15 - DNA, 23 bp, Artificial Sequence
  Synthetic sequence
tcacacgtcgctctctctaaacc

SEQ ID NO: 16 - DNA, 21 bp, Artificial Sequence
  Synthetic sequence
gtgagcgagcagaggcttaag

SEQ ID NO: 17 - DNA, 18 bp, Artificial Sequence
  Synthetic sequence
gagcccttggacggcttt

SEQ ID NO: 18 - DNA, 22 bp, Artificial Sequence
  Synthetic sequence
atgaatgcaccttcacattcct

SEQ ID NO: 19 - DNA, 21 bp, Artificial Sequence
  Synthetic sequence
tccagcagagctggaagtcga

SEQ ID NO: 20 - DNA, 20 bp, Artificial Sequence
  Synthetic sequence
ccacgtggagaaaaatggtc

SEQ ID NO: 21 - DNA, 19 bp, Artificial Sequence
  Synthetic sequence
cattgggcaggtctgtgac

SEQ ID NO: 22 - DNA, 20 bp, Artificial Sequence
  Synthetic sequence
aacacagactcgcgttgcaa

SEQ ID NO: 23 - DNA, 21 bp, Artificial Sequence
  Synthetic sequence
cggcttgtcacatctgcaagt

SEQ ID NO: 24 - DNA, 24 bp, Artificial Sequence
  Synthetic sequence
cagagtgagaccttgtctgtctcc

SEQ ID NO: 25 - DNA, 26 bp, Artificial Sequence
  Synthetic sequence
cagaagatgcatgcaacagcaccttg

SEQ ID NO: 26 - DNA, 20 bp, Artificial Sequence
  Synthetic sequence
caggctgtggctctgattgg

SEQ ID NO: 27 - DNA, 21 bp, Artificial Sequence
  Synthetic sequence
cctcacctgaaaacaggcagc

SEQ ID NO: 28 - DNA, 20 bp, Artificial Sequence
  Synthetic sequence
gcgagactgtggccttgtgt

SEQ ID NO: 29 - DNA, 21 bp, Artificial Sequence
  Synthetic sequence
cgttccagggtccacaaagtc

SEQ ID NO: 30 - RNA, 25 nt, Artificial Sequence
  Synthetic sequence
cccugcugugaugaauuacagcauu

SEQ ID NO: 31 - RNA, 25 nt, Artificial Sequence
  Synthetic sequence
ccuuuagugguccaucgccaguuau

SEQ ID NO: 32 - RNA, 19 nt, Artificial Sequence
  Synthetic sequence
  misc_feature (19)..(19): =Att
gggacuucaacgaaggaca

SEQ ID NO: 33 - protein, 9 aa, Artificial Sequence
  Synthetic sequence
YPYDVPDYA

SEQ ID NO: 34 - DNA, 19 bp, Artificial Sequence
  Synthetic sequence
tgctgggaatgctgtaatt

SEQ ID NO: 35 - DNA, 19 bp, Artificial Sequence
  Synthetic sequence
cagcgcagaagtgagcatc

SEQ ID NO: 36 - DNA, 19 bp, Artificial Sequence
  Synthetic sequence
ggatattcatggtggctgt

SEQ ID NO: 37 - DNA, 23 bp, Artificial Sequence
  Synthetic sequence
  misc_feature (21)..(21): n is a, c, g, or t
tcctcagcatcttatccgagngg

SEQ ID NO: 38 - DNA, 19 bp, Artificial Sequence
  Synthetic sequence
ccatgagcgctgctcagat

SEQ ID NO: 39 - DNA, 22 bp, Artificial Sequence
  Synthetic sequence
tcatggggttatagggaggtca

SEQ ID NO: 40 - DNA, 56 bp, Artificial Sequence
  Synthetic sequence
ctggcccctcctcagcatcttatccgagtggaaggaaatttgcgtgtggagtattt

SEQ ID NO: 41 - DNA, 55 bp, Artificial Sequence
  Synthetic sequence
ctggcccctcctcagcatcttatcgagtggaaggaaatttgcgtgtggagtattt

SEQ ID NO: 42 - DNA, 57 bp, Artificial Sequence
  Synthetic sequence
ctggcccctcctcagcatcttatccagagtggaaggaaatttgcgtgtggagtattt